European Patent Application EP 4 306 655 A1, published January 17, 2024. Title: PRIMER PROBE SET FOR HUMAN HISTAMINE RECEPTOR HRH1 MRNA DETECTION, KIT AND DETECTION METHOD. Applicant: HANGZHOU ZHEDA DIXUN BIOLOGICAL GENE ENGINEERING CO., LTD. The sequence listing filed with the application follows.

SEQUENCE LISTING (9 sequences)

SEQ ID NO: 1 - DNA, 21 bp, Artificial sequence
aatccttctctcgaacggact

SEQ ID NO: 2 - DNA, 20 bp, Artificial sequence
ggcctgtgttagacccactc

SEQ ID NO: 3 - DNA, 21 bp, Artificial sequence
ttgcctttgcctggtgctgtc

SEQ ID NO: 4 - DNA, 21 bp, Artificial sequence
gacaacagcctcaagatcatc

SEQ ID NO: 5 - DNA, 18 bp, Artificial sequence
cgccacagtttcccggag

SEQ ID NO: 6 - DNA, 24 bp, Artificial sequence
actcatgaccacagtccatgccat

SEQ ID NO: 7 - DNA, 20 bp, Artificial sequence
cagggactatgtagccgtca

SEQ ID NO: 8 - DNA, 21 bp, Artificial sequence
agagaaggattggctatcacc

SEQ ID NO: 9 - DNA, 22 bp, Artificial sequence
ctgatatctcgctggccccatg